European Patent Application EP 4 714 964 A1, published March 25, 2026. Title: peptide fragment and use thereof. Applicant: TOAGOSEI CO., LTD. The sequence listing filed with the application follows.

SEQUENCE LISTING (2 sequences)

SEQ ID NO: 1 - protein, 17 aa, synthetic construct
VLSRVVQLLREKLTRKK

SEQ ID NO: 2 - protein, 13 aa, synthetic construct
VLSRVQLREKLTR